European Patent Specification EP 3 831 948 B1, published September 6, 2023. Title: Recombinant expression vector for rapidly screening recombinant strains and application thereof. Applicant: Feed Research Institute, Chinese Academy of Agricultural Sciences. The sequence listing filed with the application follows.

SEQUENCE LISTING (22 sequences)

SEQ ID NO: 1 - DNA, 1193 bp, Trichoderma reesei
tcaacctttggcgtttccctgattcagcgtacccgtacaagtcgtaatcactattaacccagactgaccggacgtgttttgcccttcatttggagaaataatgtcattgcgatgtgtaatttgcctgcttgaccgactggggctgttcgaagcccgaatgtaggattgttatccgaactctgctcgtagaggcatgttgtgaatctgtgtcgggcaggacacgcctcgaaggttcacggcaagggaaaccaccgatagcagtgtctagtagcaacctgtaaagccgcaatgcagcatcactggaaaatacaaaccaatggctaaaagtacataagttaatgcctaaagaagtcatataccagcggctaataattgtacaatcaagtggctaaacgtaccgtaatttgccaacggcttgtggggttgcagaagcaacggcaaagccccacttccccacgtttgtttcttcactcagtccaatctcagctggtgatcccccaattgggtcgcttgtttgttccggtgaagtgaaagaagacagaggtaagaatgtctgactcggagcgttttgcatacaaccaagggcagtgatggaagacagtgaaatgttgacattcaaggagtatttagccagggatgcttgagtgtatcgtgtaaggaggtttgtctgccgatacgacgaatactgtatagtcacttctgatgaagtggtccatattgaaatgtaagtcggcactgaacaggcaaaagattgagttgaaactgcctaagatctcgggccctcgggccttcggcctttgggtgtacatgtttgtgctccgggcaaatgcaaagtgtggtaggatcgaacacactgctgcctttaccaagcagctgagggtatgtgataggcaaatgttcaggggccactgcatggtttcgaatagaaagagaagcttagccaagaacaatagccgataaagatagcctcattaaacggaatgagctagtaggcaaagtcagcgaatgtgtatatataaaggttcgaggtccgtgcctccctcatgctctccccatctactcatcaactcagatcctccaggagacttgtacaccatcttttgaggcacagaaacccaatagtcaaccgcggactgcgcatcatgtatcggaagttggccgtcatctcggccttcttggccacagctcgtgct

SEQ ID NO: 2 - DNA, 153 bp, Actiniaria
ggcggctccggctccggctccggctccagcactggtactgccactgcctccaccagcaccaacctcctcaagactggcgccgccagcaaggagcacttcagctactccctcggcggtgccgtcgtcgcggccgccatcgccgtcgctctctaa

SEQ ID NO: 3 - DNA, 675 bp, Aspergillus funigatus
atggacaacaccgaggacgtcatcaaggagttcatgcagttcaaggtgcgcatggagggctccgtgaacggccactacttcgagatcgagggcgagggcgagggcaagccctacgagggcacccagaccgccaagctgcaggtgaccaagggcggccccctgcccttcgcctgggacatcctgtccccccagttccagtacggctccaaggcctacgtgaagcaccccgccgacatccccgactacatgaagctgtccttccccgagggcttcacctgggagcgctccatgaacttcgaggacggcggcgtggtggaggtgcagcaggactcctccctgcaggacggcaccttcatctacaaggtgaagttcaagggcgtgaacttccccgccgacggccccgtaatgcagaagaagactgccggctgggagccctccaccgagaagctgtacccccaggacggcgtgctgaagggcgagatctcccacgccctgaagctgaaggacggcggccactacacctgcgacttcaagaccgtgtacaaggccaagaagcccgtgcagctgcccggcaaccactacgtggactccaagctggacatcaccaaccacaacgaggactacaccgtggtggggcagtacgagcacgccgaggcccgccactccggctcccag

SEQ ID NO: 4 - DNA, 500 bp, Trichoderma reesei
agctccgtggcgaaagcctgacgcaccggtagattcttggtgagcccgtatcatgacggcggcgggagctacatggccccgggtgatttattttttttgtatctacttctgacccttttcaaatatacggtcaactcatctttcactggagatgcggcctgcttggtattgcgatgttgtcagcttggcaaattgtggctttcgaaaacacaaaacgattccttagtagccatgcattttaagataacggaatagaagaaagaggaaattaaaaaaaaaaaaaaaacaaacatcccgttcataacccgtagaatcgccgctcttcgtgtatcccagtaccacggcaaaggtatttcatgatcgttcaatgttgatattgttcccgccagtatggctccacccccatctccgcgaatctcctcttctcgaacgcggtagtggcgcgccaattggtaatgacccatagggagacaaacagcataatagcaacagtggaaatt

SEQ ID NO: 5 - DNA, 2680 bp, Trichoderma reesei
ataaagtggcccatcgtcacctctcggcttcaactcgagtttttccctttttccttttcttcttcttcttcaaacaaagataccccccctcaacccggtgcaaccagcctggtccgaggacaaaacacgatagagctcgctgcgttggatcgctgcgcgtcttctcttgttctctctctcttttcttctctgcaacgcttataactctttttgcgcggggcatctgggaaaaccgtttcttcacacatctcttcttccacaatggctcgttcacggagctccctggccctcgggctgggcctgctctgctggatcacgctgctcttcgctcctctggcgtttgtcggaaaggccaatgccgcgagcgacgacgcggacaactacggcactgttatcggaattgtaagtcgactgacggcagcaaccccgccattttcttggtgttgatgctcaggcagccctgctaacacgcttctcctccgcccaggatctcggaactacctacagctgcgtcggtgtgatgcagaagggcaaggttgagattctcgtcaacgaccagggtaaccgaatcactccctcctacgtggcctttaccgacgaggagcgtctggttggcgattccgccaagaaccaggccgccgccaaccccaccaacaccgtctacgatgtcaagtcagttctaccgccctgttggcttctattgtataagtggacaattagctaactgttgtcacaggcgattgattggccgcaaattcgacgagaaggagatccaggccgacatcaagcacttcccctacaaggtcattgagaagaacggcaagcccgtcgtccaggtccaggtcaacggccagaagaagcagttcactcccgaggagatttctgccatgattcttggcaagatgaaggaggttgccgagtcgtacctgggcaagaaggttacccacgccgtcgtcaccgtccctgcctacttcaacgtgagtcttttccccgaaattcctcgaggattccaagagccatctgctaacagcccgataggacaaccagcgacaggccaccaaggacgccggtaccattgccggcttgaacgttctccgaatcgtcaacgaacccaccgctgccgctatcgcctatggtctggacaagaccgacggtgagcgccagatcattgtctacgatctcggtggtggtacctttgatgtttctctcctgtccattgacaatggcgtcttcgaggtcttggctaccgccggtgacacccaccttggtggtgaggactttgaccagcgcattatcaactacctggccaaggcctacaacaagaagaacaacgtcgacatctccaaggacctcaaggccatgggcaagctcaagcgtgaagccgaaaaggccaagcgtaccctctcttcccagatgagcactcgtatcgaaatcgaggccttcttcgagggcaacgacttctccgagactctcacccgggccaagttcgaggagctcaacatggacctcttcaagaagaccctgaagcctgtcgagcaggttctcaaggacgccaacgtcaagaagagcgaggttgacgacatcgttctggtcggcggttccacccgtatccccaaggttcagtctcttatcgaggagtactttaacggcaagaaggcttccaagggtatcaaccccgacgaggctgttgctttcggtgccgccgtccaggccggtgtcctttctggtgaggaaggtaccgatgacattgttctcatggacgtcaaccccctgactctcggtatcgagaccactggcggagtcatgaccaagctcattccccgcaacacccccatccccactcgcaagagccagatcttctcgactgctgccgataaccagcccgtcgtcctgatccaggtcttcgagggtgagcgttccatgaccaaggacaacaacctcctgggcaagttcgagcttaccggcattcctcctgccccccgcggtgtcccccagattgaggtttccttcgagttggatgccaacggtatcctcaaggtctccgctcacgacaagggcaccggcaagcaggagtccatcaccatcaccaacgacaagggccgtctcacccaggaggagattgaccgcatggttgccgaggccgagaagttcgccgaggaggacaaggctacccgtgagcgcatcgaggcccgtaacggtcttgagaactacgccttcagcctgaagaaccaggtcaatgacgaggagggcctcggcggcaagattgacgaggaggacaaggagactgtaagttgaagcgatccatcactgctttctgatgcggacatgtcacactaacacttgaccagattcttgacgccgtcaaggaggctaccgagtggctcgaggagaacggcgccgacgccactaccgaggactttgaggagcagaaggagaagctgtccaacgtcgcctaccccatcacctccaagatgtaccagggtgctggtggctccgaggacgatggcgacttccacgacgaattgtaaaaaattaaaaaaagggaaattattgatgcatagatacttattagaggaaccaaagaagttcccaggtgttatcgtcggttatgacgcggatgtgttttcagtcttgtaaagttcgaatgcagctctgagtgtagtagatgcataaatgaatc

SEQ ID NO: 6 - DNA, 1356 bp, Trichoderma reesei
atggcgttccagcagtcgtctcccctcgtcaagtttgaggcctctcccgccgaatccttcctctccgcccccggcgacaacttcacatccctcttcgccgactcaacaccctcaacacttaaccctcgggacatgatgacccctgacagcgtcgccgacatcgactctcgcctgtccgtcatccccgaatcacaggacgcggaagatgacgaatcacactccacatccgctaccgcaccctctacctcagaaaagaagcccgtcaagaagaggaaatcatggggccaggttcttcctgagcccaagaccaacctccctcctcgaaaacgtgcaaagacggaagatgaaaaggagcagcgccgcgtcgagcgtgttctccgcaaccgccgcgccgcgcagtcctcgcgcgagcgcaagaggctcgaggtcgaggctctcgagaagcgcaacaaggagctcgagacgctcctcatcaacgtccagaagaccaacctgatcctcgtcgaggagctcaaccgcttccgacgcagctcaggcgtcgtcacccgctcgtcctcccccctcgactctctccaggacagcatcactctctcccagcaactctttggctcgcgggatggccaaaccatgtccaaccccgagcagtccttgatggaccagatcatgagatctgccgctaaccctaccgttaacccggcctctctttccccctccctcccccccatctcggacaaggagttccagaccaaggaggaggacgaggaacaggccgacgaagatgaagagatggagcagacatggcacgagaccaaagaagccgccgccgccaaggagaagaacagcaagcagtcccgcgtctccactgattcgacacaacgtcctgcagtgtcaatcggtggagatgccgctgtccctgtcttctcagacgacgccggcgcaaactgccttggcctggaccctgttcatcaggatgatggtcctttcagcatcggccattctttcggcctgtcagcggcccttgatgcagatcgctatctcctcgaaagccaacttctcgcttcgcccaacgcctcaactgttgacgacgattatctggctggtgactctgccgcctgcttcacgaatcctctcccctccgactacgacttcgacatcaacgacttcctcacagacgacgcaaaccacgccgcctatgacattgtggcagcgagcaactatgccgctgcggaccgcgagctcgacctcgagatccacgaccctgagaatcagatcccttcgcgacattctatccagcagccccagtctggcgcgtcctctcatggatgcgacgatggcggcattgcggttggtgtctga

SEQ ID NO: 7 - DNA, 2919 bp, Trichoderma reesei
gactgacccccccggttgggcccctcgtcccgtctccaacagagcaccaccagacaaagacccctgcccgcgcgaatccagacccccccagcaattccgggcctcgttgatcctcctctactgtagttgtacatacatacctaccgactgcattgcattggtacagctgcaggcacttccaggcacggccaccaaattgcagcggcccttgcttgcttgcttggttcgagaactaggatctgtgtcttttgccttgccttgtcttgtctgggttcctgctcgtctgcggcaatcggaacgccgccagtgcggtgccaagcaaaccagccaaggtaggtacctaccactaggcttcttttctcgttgtctcactctctcttttcctctttgtcctctcttatccccatcttttctctctctctctgctcctttcctaaccacttccctacctttctctttttccttttcttgtcatctccatcttggctgacgaaaaaggtctgactgggtaggtattatctggcagacttgtgtgtatcattcaccctatttctgcttcatagtacatgtactgtacctgaacggctcaaccgctatttacgactcttatttttttgtggcgttggtcacgtttgccagctgttgtccgtctttctagggctcctcaaacttgacctgaccgagctccctttctggacccggtgggcttcacttccagctgctgagcgacctgagccgaacatcctcagtccttgtccagcgcaattcattttctttccttttctttttttttattcctttctttacttttattctctctttttctcctcttcctcttcttcttctttctcctcctcctccatatcctcactctcgtctccctcattactaccctctcggctcctcaggtccaccaaccctcccgcacccaaacctctgccgctgaaacccattcggtggtcgccgttttttttttttttttctcacccccaaagtcgcaatatcgggtatcgccgccggcattgaatcgccttctccgctagcatcgactactgctgctctgctctcgttgccagcgctgctccctagaattttgaccaggggacgagcccgacattaaagcaactccctcgcctcgagacgactcggatcgcacgaaattctcccaatcgccgacagttcctactcctcttcctcccgcacggctgtcgcgcttccaacgtcattcgcacagcagaattgtgccatctctctcttttttttccccccctctaaaccgccacaacggcaccctaagggttaaactatccaaccagccgcagcctcagcctctctcagcctcatcagccatggcaccacacccgacgctcaaggccaccttcgcggccaggagcgagacggcgacgcacccgctgacggcttacctgttcaagctcatggacctcaaggcgtccaacctgtgcctgagcgccgacgtgccgacagcgcgcgagctgctgtacctggccgacaagattggcccgtcgattgtcgtgctcaagacgcactacgacatggtctcgggctgggacttccacccggagacgggcacgggagcccagctggcgtcgctggcgcgcaagcacggcttcctcatcttcgaggaccgcaagtttggcgacattggccacaccgtcgagctgcagtacacgggcgggtcggcgcgcatcatcgactgggcgcacattgtcaacgtcaacatggtgcccggcaaggcgtcggtggcctcgctggcccagggcgccaagcgctggctcgagcgctacccctgcgaggtcaagacgtccgtcaccgtcggcacgcccaccatggactcgtttgacgacgacgccgactccagggacgccgagcccgccggcgccgtcaacggcatgggctccattggcgtcctggacaagcccatccactcgaaccggtccggcgacggccgcaagggcagcatcgtctccatcaccaccgtcacccagcagtacgagtccgtctcctcgccccggttaacaaaggccatcgccgagggcgacgagtcgctcttcccgggcatcgaggaggcgccgctgagccgcggcctcctgatcctcgcccaaatgtccagccagggcaacttcatgaacaaggagtacacgcaggcctgcgtcgaggccgcccgggagcacaaggactttgtcatgggcttcatctcgcaggagacgctcaacaccgagcccgacgatgcctttatccacatgacgcccggctgccagctgccccccgaagacgaggaccagcagaccaacggatcggtcggtggagacggccagggccagcagtacaacacgccgcacaagctgattggcatcgccggtagcgacattgccattgtgggccggggcatcctcaaggcctcagaccccgtagaggaggcagagcggtaccgatcagcagcgtggaaagcctacaccgagaggctgctgcgataggggagggaagggaagaaagaagtaaagaaaggcatttagcaagaagggggaaaagggagggaggacaaacggagctgagaaagagctcttgtccaaagcccggcatcatagaatgcagctgtatttaggcgacctctttttccatcttgtcgatttttgttatgacgtaccagttgggatgatggatgattgtaccccagctgcgattgatgtgtatctttgcatgcaacaacacgcgatggcggaggcgaactgcacattggaaggttcatatatggtcctgacatatctggtggatctggaagcatggaattgtatttttgatttggcatttgcttttgcgcgtggagggaacatatcaccctcgggcatttttcatttggtaggatggtttggatgcagttgatcgataagcttgatatcg

SEQ ID NO: 8 - DNA, 20 bp, Artificial Sequence
  synthesized primer
gttgagggggggtatctttg

SEQ ID NO: 9 - DNA, 20 bp, Artificial Sequence
  synthesized primer
gttgagggggggtatctttg

SEQ ID NO: 10 - DNA, 20 bp, Artificial Sequence
  synthesized primer
ttgagtcggcgaagagggat

SEQ ID NO: 11 - DNA, 20 bp, Artificial Sequence
  synthesized primer
ctcctccctctctccctctc

SEQ ID NO: 12 - DNA, 20 bp, Artificial Sequence
  synthesized primer
tcgcatcaggtaagctgttg

SEQ ID NO: 13 - DNA, 20 bp, Artificial Sequence
  synthesized primer
gcaatcaagcgacggaggac

SEQ ID NO: 14 - DNA, 20 bp, Artificial Sequence
  synthesized primer
agagtgtcgtcaccagtata

SEQ ID NO: 15 - DNA, 20 bp, Artificial Sequence
  synthesized primer
gacgggagggaggatacgta

SEQ ID NO: 16 - DNA, 20 bp, Artificial Sequence
  synthesized primer
aaggagccatctctactgcg

SEQ ID NO: 17 - DNA, 20 bp, Artificial Sequence
  synthesized primer
tgagagcggtggtatccacg

SEQ ID NO: 18 - DNA, 25 bp, Artificial Sequence
  synthesized primer
ggtaccaccagacatgacaatgttg

SEQ ID NO: 19 - DNA, 20 bp, Artificial Sequence
  synthesized primer
acaacgtcctgcagtgtcaa

SEQ ID NO: 20 - DNA, 20 bp, Artificial Sequence
  synthesized primer
tagcgatctgcatcaagggc

SEQ ID NO: 21 - DNA, 19 bp, Artificial Sequence
  synthesized primer
aagaaggttacccacgccg

SEQ ID NO: 22 - DNA, 21 bp, Artificial Sequence
  synthesized primer
atcaaaggtaccaccaccgag